European Patent Application EP 4 530 292 A1, published April 2, 2025. Title: 바이러스 뉴클레오캡시드를 이용한 결정성 단백질 기반 목적 단백질 융합 자가 조립 나노 입자 제조 플랫폼. Applicant: 주식회사 백스다임. The sequence listing filed with the application follows.

SEQUENCE LISTING (13 sequences)

SEQ ID NO: 1 - skipped

SEQ ID NO: 2 - DNA, 162 bp, Human immunodeficiency virus 1
  source 1..162: mol_type = genomic DNA
cagcggggaaacttcaggaaccagagaaaaactgtgaagtgcttcaattgcggaaaggagggccacatcgctaagaactgccgcgcccccagaaagaaaggctgctggagatgcggcagagagggccaccagatgaaggactgcacagagagacaggcaaac

SEQ ID NO: 3 - DNA, 162 bp, synthetic construct
  source 1..162: mol_type = other DNA
cagcgtggtaacttccgtaaccagcgtaaaaccgttaaatgcttcaactgcggcaaagaaggccacatcgcgaaaaactgccgtgcgccgcgtaaaaaaggctgctggcgttgcggccgtgaaggccaccagatgaaagattgcaccgaacgtcaggcgaac

SEQ ID NO: 4 - protein, 264 aa, Mycobacterium tuberculosis
NNLYRDLAPVTEAAWAEIELEAARTFKRHIAGRRVVDVSDPGGPVTAAVSTGRLIDVKAPTNGVIAHLRASKPLVRLRVPFTLSRNEIDDVERGSKDSDWEPVKEAAKKLAFVEDRTIFEGYSAASIEGIRSASSNPALTLPEDPREIPDVISQALSELRLAGVDGPYSVLLSADVYTKVSETSDHGYPIREHLNRLVDGDIIWAPAIDGAFVLTTRGGDFDLQLGTDVAIGYASHDTDTVRLYLQETLTFLCYTAEASVALSH

SEQ ID NO: 5 - DNA, 792 bp, Mycobacterium tuberculosis
  source 1..792: mol_type = genomic DNA
aataacctgtaccgggaccttgcaccagtcactgaggctgcgtgggccgagatcgagcttgaggccgcacgtacgtttaagcgtcatattgcgggccgtcgggttgtggatgtatcagatcctggaggtcctgtaaccgctgcggtatcgacagggcgtttgattgacgtaaaggctccaaccaacggtgtcattgcccacttacgcgccagcaagcctttagttcgtttaagagtgccctttacgttaagccggaacgaaattgatgatgtggaacgtgggtcaaaggacagtgattgggaaccagtgaaagaggcggcgaagaagttggccttcgtcgaagatcgtaccatatttgaaggctactccgctgcttccatagaagggattcggtccgcctcctcaaatccagcattaacgctgcctgaagacccgcgcgagattcctgatgtaatctcacaggcactttcggaattacgtttggcaggggtcgatggaccatacagtgttcttttgagtgcagatgtatacaccaaggtgagcgagaccagtgatcacggctatccaatacgggaacacctgaacagacttgtcgatggcgacataatctgggcgcccgcaattgacggcgcattcgtgttgaccacccgtggtggtgattttgatttacaattaggcaccgatgttgcgattgggtatgcgagtcatgatacggacactgtacgtttgtatcttcaagagacgctgacgttcttatgttacaccgctgaggcgtccgtggcgctttcgcat

SEQ ID NO: 6 - protein, 157 aa, Escherichia coli
KGDTKVINYLNKLLGNELVAINQYFLHARMFKNWGLKRLNDVEYHESIDEMKHADRYIERILFLEGLPNLQDLGKLNIGEDVEEMLRSDLALELDGAKNLREAIGYADSVHDYVSRDMMIEILRDEEGHIDWLETELDLIQKMGLQNYLQAQIREEG

SEQ ID NO: 7 - DNA, 471 bp, Escherichia coli
  source 1..471: mol_type = genomic DNA
aaaggtgatactaaagttataaattatctcaacaaactgttgggaaatgagcttgtcgcaatcaatcagtactttctccatgcccgaatgtttaaaaactggggtctcaaacgtctcaatgatgtggagtatcatgaatccattgatgagatgaaacacgccgatcgttatattgagcgcattctttttctggaaggtcttccaaacttacaggacctgggcaaactgaacattggtgaagatgttgaggaaatgctgcgttctgatctggcacttgagctggatggcgcgaagaatttgcgtgaggcaattggttatgccgatagcgttcatgattacgtcagccgcgatatgatgatagaaattttgcgtgatgaagaaggccatatcgactggctggaaacggaacttgatctgattcagaagatgggcctgcaaaattatctgcaagcacagatccgcgaagaaggt

SEQ ID NO: 8 - DNA, 1023 bp, synthetic construct
  source 1..1023: mol_type = other DNA
atgcagcggggaaacttcaggaaccagagaaaaactgtgaagtgcttcaattgcggaaaggagggccacatcgctaagaactgccgcgcccccagaaagaaaggctgctggagatgcggcagagagggccaccagatgaaggactgcacagagagacaggcaaaccatcaccatcaccatcacgaaaacctgtattttcagggtggatccaataacctgtaccgggaccttgcaccagtcactgaggctgcgtgggccgagatcgagcttgaggccgcacgtacgtttaagcgtcatattgcgggccgtcgggttgtggatgtatcagatcctggaggtcctgtaaccgctgcggtatcgacagggcgtttgattgacgtaaaggctccaaccaacggtgtcattgcccacttacgcgccagcaagcctttagttcgtttaagagtgccctttacgttaagccggaacgaaattgatgatgtggaacgtgggtcaaaggacagtgattgggaaccagtgaaagaggcggcgaagaagttggccttcgtcgaagatcgtaccatatttgaaggctactccgctgcttccatagaagggattcggtccgcctcctcaaatccagcattaacgctgcctgaagacccgcgcgagattcctgatgtaatctcacaggcactttcggaattacgtttggcaggggtcgatggaccatacagtgttcttttgagtgcagatgtatacaccaaggtgagcgagaccagtgatcacggctatccaatacgggaacacctgaacagacttgtcgatggcgacataatctgggcgcccgcaattgacggcgcattcgtgttgaccacccgtggtggtgattttgatttacaattaggcaccgatgttgcgattgggtatgcgagtcatgatacggacactgtacgtttgtatcttcaagagacgctgacgttcttatgttacaccgctgaggcgtccgtggcgctttcgcatgatatcgtcgacaagctttga

SEQ ID NO: 9 - protein, 340 aa, synthetic construct
MQRGNFRNQRKTVKCFNCGKEGHIAKNCRAPRKKGCWRCGREGHQMKDCTERQANHHHHHHENLYFQGGSNNLYRDLAPVTEAAWAEIELEAARTFKRHIAGRRVVDVSDPGGPVTAAVSTGRLIDVKAPTNGVIAHLRASKPLVRLRVPFTLSRNEIDDVERGSKDSDWEPVKEAAKKLAFVEDRTIFEGYSAASIEGIRSASSNPALTLPEDPREIPDVISQALSELRLAGVDGPYSVLLSADVYTKVSETSDHGYPIREHLNRLVDGDIIWAPAIDGAFVLTTRGGDFDLQLGTDVAIGYASHDTDTVRLYLQETLTFLCYTAEASVALSHDIVDKL

SEQ ID NO: 10 - DNA, 1620 bp, synthetic construct
  source 1..1620: mol_type = other DNA
cagcggggaaacttcaggaaccagagaaaaactgtgaagtgcttcaattgcggaaaggagggccacatcgctaagaactgccgcgcccccagaaagaaaggctgctggagatgcggcagagagggccaccagatgaaggactgcacagagagacaggcaaacgaaaacctgtattttcagggccatcaccatcaccatcacgatgatgatgatggtaccggatccaataacctgtaccgggaccttgcaccagtcactgaggctgcgtgggccgagatcgagcttgaggccgcacgtacgtttaagcgtcatattgcgggccgtcgggttgtggatgtatcagatcctggaggtcctgtaaccgctgcggtatcgacagggcgtttgattgacgtaaaggctccaaccaacggtgtcattgcccacttacgcgccagcaagcctttagttcgtttaagagtgccctttacgttaagccggaacgaaattgatgatgtggaacgtgggtcaaaggacagtgattgggaaccagtgaaagaggcggcgaagaagttggccttcgtcgaagatcgtaccatatttgaaggctactccgctgcttccatagaagggattcggtccgcctcctcaaatccagcattaacgctgcctgaagacccgcgcgagattcctgatgtaatctcacaggcactttcggaattacgtttggcaggggtcgatggaccatacagtgttcttttgagtgcagatgtatacaccaaggtgagcgagaccagtgatcacggctatccaatacgggaacacctgaacagacttgtcgatggcgacataatctgggcgcccgcaattgacggcgcattcgtgttgaccacccgtggtggtgattttgatttacaattaggcaccgatgttgcgattgggtatgcgagtcatgatacggacactgtacgtttgtatcttcaagagacgctgacgttcttatgttacaccgctgaggcgtccgtggcgctttcgcatgatatcgtcgacaacataacaaatctatgtccctttggagaagtgtttaacgcgacccgttttgccagcgtttacgcatggaatcgcaagcgcatttctaactgcgtggcggactacagcgtgctgtataattccgcgtcgttctctacgtttaaatgctacggcgtgagcccgactaagttgaatgatctgtgttttaccaatgtttacgctgacagctttgttattcgtggtgatgaggttcgtcagattgcgccaggtcagaccggtaaaatcgcggactataactacaaacttccggatgatttcaccggctgcgtcatcgcctggaactccaacaacttggactcgaaggtgggtggtaattacaactacctcagacgtctgttccgcaagtctaacctgaaaccgtttgaacgtgacatcagcaccgagatctaccaagcgggtagcaccccgtgtaatggcgttgaaggtttcaactgctatttcccgctgcagagctatggcttccaaccgacgaacggcgtgggctatcaaccgtatcgtgttgtcgtactgagcttcgagaacaagtccgctccggcaaccgtttgcggtccg

SEQ ID NO: 11 - protein, 540 aa, synthetic construct
QRGNFRNQRKTVKCFNCGKEGHIAKNCRAPRKKGCWRCGREGHQMKDCTERQANENLYFQGHHHHHHDDDDGTGSNNLYRDLAPVTEAAWAEIELEAARTFKRHIAGRRVVDVSDPGGPVTAAVSTGRLIDVKAPTNGVIAHLRASKPLVRLRVPFTLSRNEIDDVERGSKDSDWEPVKEAAKKLAFVEDRTIFEGYSAASIEGIRSASSNPALTLPEDPREIPDVISQALSELRLAGVDGPYSVLLSADVYTKVSETSDHGYPIREHLNRLVDGDIIWAPAIDGAFVLTTRGGDFDLQLGTDVAIGYASHDTDTVRLYLQETLTFLCYTAEASVALSHDIVDNITNLCPFGEVFNATRFASVYAWNRKRISNCVADYSVLYNSASFSTFKCYGVSPTKLNDLCFTNVYADSFVIRGDEVRQIAPGQTGKIADYNYKLPDDFTGCVIAWNSNNLDSKVGGNYNYLRRLFRKSNLKPFERDISTEIYQAGSTPCNGVEGFNCYFPLQSYGFQPTNGVGYQPYRVVVLSFENKSAPATVCGP

SEQ ID NO: 12 - DNA, 1371 bp, synthetic construct
  source 1..1371: mol_type = other DNA
cagcggggaaacttcaggaaccagagaaaaactgtgaagtgcttcaattgcggaaaggagggccacatcgctaagaactgccgcgcccccagaaagaaaggctgctggagatgcggcagagagggccaccagatgaaggactgcacagagagacaggcaaaccatcatcatcatcatcatgaaaacctgtattttcagggtggtaccggatccggagtgaagcctctaattttaagagattgtagtgtagctggatggctcctcgggaacccaatgtgtgacgaattcatcaatgtaccggaatggtcttacatagtggagaaggccaatccaaccaatgacctctgttacccagggagtttcaacgactatgaagaactgaaacacctattgagcagaataaaccattttgagaaaattcaaatcatccccaaaagttcttggtccgatcatgaagcctcatcaggagtgagctcagcatgtccatacctgggaagtccctccttttttagaaatgtggtatggcttatcaaaaagaacagtacatacccaacaataaagaaaagctacaataataccaaccaagaagatcttttggtactgtggggaattcaccatcctaatgatgcggcagagcagacaaggctatatcaaaacccaaccacctatatttccattgggacatcaacactaaaccagagattggtaccaaaaatagctactagatccaaagtaaacgggcaaagtggaaggatggagttcttctggacaattttaaaacctaatgatgcaatcaacttcgagagtaatggaaatttcattgctccagaatatgcatacaaaattgtcaagaaaggggactcagcaattatgaaaagtgaattggatatcgtcgacatgaaaggtgatactaaagttataaattatctcaacaaactgttgggaaatgagcttgtcgcaatcaatcagtactttctccatgcccgaatgtttaaaaactggggtctcaaacgtctcaatgatgtggagtatcatgaatccattgatgagatgaaacacgccgatcgttatattgagcgcattctttttctggaaggtcttccaaacttacaggacctgggcaaactgaacattggtgaagatgttgaggaaatgctgcgttctgatctggcacttgagctggatggcgcgaagaatttgcgtgaggcaattggttatgccgatagcgttcatgattacgtcagccgcgatatgatgatagaaattttgcgtgatgaagaaggccatatcgactggctggaaacggaacttgatctgattcagaagatgggcctgcaaaattatctgcaagcacagatccgcgaagaaggt

SEQ ID NO: 13 - protein, 457 aa, synthetic construct
QRGNFRNQRKTVKCFNCGKEGHIAKNCRAPRKKGCWRCGREGHQMKDCTERQANHHHHHHENLYFQGGTGSGVKPLILRDCSVAGWLLGNPMCDEFINVPEWSYIVEKANPTNDLCYPGSFNDYEELKHLLSRINHFEKIQIIPKSSWSDHEASSGVSSACPYLGSPSFFRNVVWLIKKNSTYPTIKKSYNNTNQEDLLVLWGIHHPNDAAEQTRLYQNPTTYISIGTSTLNQRLVPKIATRSKVNGQSGRMEFFWTILKPNDAINFESNGNFIAPEYAYKIVKKGDSAIMKSELDIVDMKGDTKVINYLNKLLGNELVAINQYFLHARMFKNWGLKRLNDVEYHESIDEMKHADRYIERILFLEGLPNLQDLGKLNIGEDVEEMLRSDLALELDGAKNLREAIGYADSVHDYVSRDMMIEILRDEEGHIDWLETELDLIQKMGLQNYLQAQIREEG